European Patent Application EP 4 678 753 A1, published January 14, 2026. Title: PREPARATION METHOD FOR ANTIGENIC EPITOPE. Applicant: GUANGZHOU MEDICAL UNIVERSITY. The sequence listing filed with the application follows.

SEQUENCE LISTING (28 sequences)

SEQ ID NO: 1 - protein, 9 aa, synthetic construct
LPYLGWLVF

SEQ ID NO: 2 - RNA, 27 nt, synthetic construct
  source 1..27: mol_type = other RNA
ctgccttatctagggtggctggtcttc

SEQ ID NO: 3 - protein, 9 aa, synthetic construct
LPCLGWLVF

SEQ ID NO: 4 - RNA, 27 nt, synthetic construct
  source 1..27: mol_type = other RNA
ctgccttgtctagggtggctggtcttc

SEQ ID NO: 5 - DNA, 63 bp, synthetic construct
  source 1..63: mol_type = other DNA
aacatgaggatcacccatgtcctagacaaggcagaatttcttaacatgaggatcacccatgtc

SEQ ID NO: 6 - DNA, 151 bp, synthetic construct
  source 1..151: mol_type = other DNA
tcataaagggcgtctatgaacatctggagcgccagaaaacttgttgtgacaacagcgaagaccagccaccctagacaaggcagaatttcttccagggagtaccggtgcaataaattgcacctattcccatcaccgtcaccacctgagccac

SEQ ID NO: 7 - DNA, 84 bp, synthetic construct
  source 1..84: mol_type = other DNA
cagcgaagacggccctgaaaaagggccccaccctagacaaggcagaatttcttccagggccctgaaaaagggccgtaccggtgc

SEQ ID NO: 8 - DNA, 24 bp, synthetic construct
  source 1..24: mol_type = other DNA
tgataacaagaagccagacaaagc

SEQ ID NO: 9 - DNA, 23 bp, synthetic construct
  source 1..23: mol_type = other DNA
ccaggaaattagggtcgtggaag

SEQ ID NO: 10 - protein, 9 aa, synthetic construct
VYKDQISVL

SEQ ID NO: 11 - protein, 9 aa, synthetic construct
VYKDQMSVL

SEQ ID NO: 12 - DNA, 63 bp, synthetic construct
  source 1..63: mol_type = other DNA
aacatgaggatcacccatgtcactgacatttgatctttgtacaacatgaggatcacccatgtc

SEQ ID NO: 13 - DNA, 21 bp, synthetic construct
  source 1..21: mol_type = other DNA
gcagaagaagcaactgaagcc

SEQ ID NO: 14 - DNA, 21 bp, synthetic construct
  source 1..21: mol_type = other DNA
tgcaagacaccataagagctg

SEQ ID NO: 15 - protein, 9 aa, synthetic construct
FMNKFIYEI

SEQ ID NO: 16 - protein, 9 aa, synthetic construct
FMNKFVYEI

SEQ ID NO: 17 - protein, 9 aa, synthetic construct
FMNKFICEI

SEQ ID NO: 18 - protein, 9 aa, synthetic construct
FMNRFIYEI

SEQ ID NO: 19 - DNA, 151 bp, synthetic construct
  source 1..151: mol_type = other DNA
atagcgagcagcccaaagaagaattgtaggtgcatacaggaagggatgccttcttgctatctcataaatgaatctgttcatgaatgtctccctgtcttcttcatatgcttcacagcttgtgacaggttctggaacttggaaaagtgggatc

SEQ ID NO: 20 - DNA, 63 bp, synthetic construct
  source 1..63: mol_type = other DNA
aacatgaggatcacccatgtctgaatctgttcatgaatgtctaacatgaggatcacccatgtc

SEQ ID NO: 21 - DNA, 84 bp, synthetic construct
  source 1..84: mol_type = other DNA
ttcttgctatggccctgaaaaagggccataaatgaatctgttcatgaatgtctccctggccctgaaaaagggccttcttcatat

SEQ ID NO: 22 - DNA, 22 bp, synthetic construct
  source 1..22: mol_type = other DNA
cagccaaagtgaagagggaaga

SEQ ID NO: 23 - DNA, 22 bp, synthetic construct
  source 1..22: mol_type = other DNA
ttttccccatcctgcagacaat

SEQ ID NO: 24 - DNA, 2780 bp, synthetic construct
  source 1..2780: mol_type = other DNA
gaattcgagggcctatttcccatgattccttcatatttgcatatacgatacaaggctgttagagagataattagaattaatttgactgtaaacacaaagatattagtacaaaatacgtgacgtagaaagtaataatttcttgggtagtttgcagttttaaaattatgttttaaaatggactatcatatgcttaccgtaacttgaaagtatttcgatttcttggctttatatatcttgtggaaaggacgaaacaccgaacatgaggatcacccatgtcggagacggaccgtctccaacatgaggatcacccatgtctttttttaagcttggcgtaatcatgacgcgttgacattgattattgactagttattaatagtaatcaattacggggtcattagttcatagcccatatatggagttccgcgttacataacttacggtaaatggcccgcctggctgaccgcccaacgacccccgcccattgacgtcaataatgacgtatgttcccatagtaacgccaatagggactttccattgacgtcaatgggtggagtatttacggtaaactgcccacttggcagtacatcaagtgtatcatatgccaagtacgccccctattgacgtcaatgacggtaaatggcccgcctggcattatgcccagtacatgaccttatgggactttcctacttggcagtacatctacgtattagtcatcgctattaccatggtgatgcggttttggcagtacatcaatgggcgtggatagcggtttgactcacggggatttccaagtctccaccccattgacgtcaatgggagtttgttttggcaccaaaatcaacgggactttccaaaatgtcgtaacaactccgccccattgacgcaaatgggcggtaggcgtgtacggtgggaggtctatataagcagagctctctggctaactagagaacccactgcttactggcttatcgaaattaatacgactcactatagggagacccaagctggctagcgccaccatggcgtctaatttcacccagttcgtgctcgtggacaacggcggcaccggcgacgtgaccgtggccccttccaacttcgccaacggcatagctgagtggatcagcagcaacagcaggtctcaggcctacaaagtgacctgcagcgttagacagagcagcgcccagaaccggaagtacaccatcaaggtggaggtgcccaaaggcgcctggcggagctatctgaacatggaactgaccatccctatcttcgctacaaattccgattgtgaattgatcgtgaaggctatgcagggcctgctgaaggacggcaatcccatccctagcgccatcgccgccaattcgggcatctacggcggaagcggctctggcgccggctctggttctcctgccggaggcggcgcccctggctccggcggcggtagcaaggccgaacggatgggcttcaccgaggtgacccctgtgacaggcgcttctctgcggagaaccatgctgctgctgagccggtctccagaagctcagcctaagaccctgccactgacaggatctacattccatgatcagatcgccatgctgagccacagatgtttcaacaccctgaccaactcctttcagcccagcctgctgggcagaaagatcctggcagccatcattatgaaaaaggacagcgaggacatgggcgtcgtggtcagcctgggcactggcaacagatgcgtgaagggcgattcgctgtccctgaagggagaaaccgtgaacgactgccacgccgagatcatttcaagacggggcttcatccggtttctgtacagcgagctgatgaaatacaacagccaaaccgccaaggacagcatcttcgagcctgccaaggggggagagaagctgcagatcaagaaaaccgtgagcttccacctgtacatcagcacggccccttgtggcgacggcgccctgttcgacaagagctgctctgatagagccatggaaagcacagagagcagacactaccctgtgtttgagaaccctaagcaggggaagctgcgtacaaaggtggaaaacggccagggcaccatccccgtggaaagctctgatatcgtgcccacatgggacggcatcagactgggcgagagactgagaaccatgagctgcagcgacaagatcctgagatggaacgtgctgggactgcaaggagccctgctgacccacttcctgcagcctatctacctgaagagcgtgaccctgggctacctcttttctcagggccacctgacccgggccatttgctgccgggtgactagagatggaagcgctttcgaggacggcctgcggcaccccttcatcgtgaaccacccaaaggttggaagagtgtccatctacgactccaaaagacaaagcggaaagaccaaggagacatcagtgaactggtgcctggccgacggctatgatctggaaatcctggacggcacaagaggcaccgtcgacggcccccggaacgagctgagcagagtgagcaagaagaacatcttcctgctgttcaagaagctgtgtagctttagatacagacgcgacctgctgcgcctgtcttatggcgaggccaagaaagccgctagagactacgaaacagccaagaactacttcaagaaaggcctgaaggatatgggatacggcaattggatcagcaaacctcaggaggaaaagaatttctacctgtgccccgtgggcagcggttccggcagcctgcctcctctcgaaagactgacactgggatcc

SEQ ID NO: 25 - DNA, 332 bp, synthetic construct
  source 1..332: mol_type = other DNA
gaattcgagggcctatttcccatgattccttcatatttgcatatacgatacaaggctgttagagagataattagaattaatttgactgtaaacacaaagatattagtacaaaatacgtgacgtagaaagtaataatttcttgggtagtttgcagttttaaaattatgttttaaaatggactatcatatgcttaccgtaacttgaaagtatttcgatttcttggctttatatatcttgtggaaaggacgaaacaccgaacatgaggatcacccatgtcctagacaaggcagaatttcttaacatgaggatcacccatgtctttttttaagctt

SEQ ID NO: 26 - DNA, 1389 bp, synthetic construct
  source 1..1389: mol_type = other DNA
gctagcgccaccatggctccaaaaaagaagagaaaggtagatccaaaaaagaagagaaaggtagatccaaaaaagaagagaaaggtaggcagcacctccggagtaaacgcacgaacacgacgacgtgagcgtcgcgctgagaaacaagctcaatggaaagctgcaaacttgcacttggatcagacgccatctcgccagcctattcccagtgagggtcttcagctgcatttaccgcaggttttagctgacgctgtctcacgcctggtcctgggtaagtttggtgacctgaccgacaacttctcctcccctcacgctcgcagaaaagtgctggctggagtcgtcatgacaacaggcacagatgttaaagatgccaaggtgataagtgtttctacaggaacaaaatgtattaatggtgaatacatgagtgatcgtggccttgcattaaatgactgccatgcagaaataatatctcggagatccttgctcagatttctttatacacaacttgagctttacttaaataacaaagatgatcaaaaaagatccatctttcagaaatcagagcgaggggggtttaggctgaaggagaatgtccagtttcatctgtacatcagcacctctccctgtggagatgccagaatcttctcaccacatgagccaatcctggaagaaccagcagatagacacccaaatcgtaaagcaagaggacagctacggaccaaaatagagtctggtcaggggacgattccagtgcgctccaatgcgagcatccaaacgtgggacggggtgctgcaaggggagcggctgctcaccatgtcctgcagtgacaagattgcacgctggaacgtggtgggcatccagggatccctgctcagcattttcgtggagcccatttacttctcgagcatcatcctgggcagcctttaccacggggaccacctttccagggccatgtaccagcggatctccaacatagaggacctgccacctctctacaccctcaacaagcctttgctcagtggcatcagcaatgcagaagcacggcagccagggaaggcccccaacttcagtgtcaactggacggtaggcgactccgctattgaggtcatcaacgccacgactgggaaggatgagctgggccgcgcgtcccgcctgtgtaagcacgcgttgtactgtcgctggatgcgtgtgcacggcaaggttccctcccacttactacgctccaagattaccaaacccaacgtgtaccatgagtccaagctggcggcaaaggagtaccaggccgccaaggcgcgtctgttcacagccttcatcaaggcggggctgggggcctgggtggagaagcccaccgagcaggaccagttctcactcacgccactagtcggatcc

SEQ ID NO: 27 - DNA, 1480 bp, synthetic construct
  source 1..1480: mol_type = other DNA
gctagccgccaccatgtctgataacaagaagccagacaaagcccacagtggctcaggtggtgacggtgatgggaataggtgcaatttattgcaccggtactccctggaagaaattctgccttatctagggtggctggtcttcgctgttgtcacaacaagttttctggcgctccagatgttcatagacgccctttatgaggagcagtatgaaagggatgtggcctggatagccaggcaaagcaagcgcatgtcctctgtcgatgaggatgaagacgatgaggatgatgaggatgactactacgacgacgaggacgacgacgacgatgccttctatgatgatgaggatgatgaggaagaagaattggagaacctgatggatgatgaatcagaagatgaggccgaagaagagatgagcgtggaaatgggtgccggagctgaggaaatgggtgctggcgctaactgtgcctgtgttcctggccatcatttaaggaagaatgaagtgaagtgtaggatgatttatttcttccacgaccctaatttcctggtgtctataccagtgaaccctaaggaacaaatggagtgtaggtgtgaaaatgctgatgaagaggttgcaatggaagaggaagaagaagaagaggaggaggaggaggaagaggaaatgggaaacccggatggcttctcacctggatccggaagcggagctactaacttcagcctgctgaagcaggctggagacgtggaggagaaccctggacctatgagcaagggcgaggagctgttcaccggggtggtgcccatcctggtcgagctggacggcgacgtaaacggccacaagttcagcgtgtccggcgagggcgagggcgatgccacctacggcaagctgaccctgaagttcatctgcaccaccggcaagctgcccgtgccctggcccaccctcgtgaccaccctgacctacggcgtgcagtgcttcagccgctaccccgaccacatgaagcagcacgacttcttcaagtccgccatgcccgaaggctacgtccaggagcgcaccatcttcttcaaggacgacggcaactacaagacccgcgccgaggtgaagttcgagggcgacaccctggtgaaccgcatcgagctgaagggcatcgacttcaaggaggacggcaacatcctggggcacaagctggagtacaactacaacagccacaacgtctatatcatggccgacaagcagaagaacggcatcaaggtgaacttcaagatccgccacaacatcgaggacggcagcgtgcagctcgccgaccactaccagcagaacacccccatcggcgacggccccgtgctgctgcccgacaaccactacctgagcacccagtccgccctgagcaaagaccccaacgagaagcgcgatcacatggtcctgctggagttcgtgaccgccgccgggatcactcacggcatggacgagctgtacaagtaagtcgac

SEQ ID NO: 28 - DNA, 2625 bp, synthetic construct
  source 1..2625: mol_type = other DNA
ctagccgccaccatgaagtgggtggaatcaatttttttaattttcctactaaattttactgaatccagaacactgcatagaaatgaatatggaatagcttccatattggattcttaccaatgtactgcagagataagtttagctgacctggctaccatattttttgcccagtttgttcaagaagccacttacaaggaagtaagcaaaatggtgaaagatgcattgactgcaattgagaaacccactggagatgaacagtcttcagggtgtttagaaaaccagctacctgcctttctggaagaactttgccatgagaaagaaattttggagaagtacggacattcagactgctgcagccaaagtgaagagggaagacataactgttttcttgcacacaaaaagcccactccagcatcgatcccacttttccaagttccagaacctgtcacaagctgtgaagcatatgaagaagacagggagacattcatgaacaaattcatttatgagatagcaagaaggcatcccttcctgtatgcacctacaattcttctttgggctgctcgctatgacaaaataattccatcttgctgcaaagctgaaaatgcagttgaatgcttccaaacaaaggcagcaacagttacaaaagaattaagagaaagcagcttgttaaatcaacatgcatgtgcagtaatgaaaaattttgggacccgaactttccaagccataactgttactaaactgagtcagaagtttaccaaagttaattttactgaaatccagaaactagtcctggatgtggcccatgtacatgagcactgttgcagaggagatgtgctggattgtctgcaggatggggaaaaaatcatgtcctacatatgttctcaacaagacactctgtcaaacaaaataacagaatgctgcaaactgaccacgctggaacgtggtcaatgtataattcatgcagaaaatgatgaaaaacctgaaggtctatctccaaatctaaacaggtttttaggagatagagattttaaccaattttcttcaggggaaaaaaatatcttcttggcaagttttgttcatgaatattcaagaagacatcctcagcttgctgtctcagtaattctaagagttgctaaaggataccaggagttattggagaagtgtttccagactgaaaaccctcttgaatgccaagataaaggagaagaagaattacagaaatacatccaggagagccaagcattggcaaagcgaagctgcggcctcttccagaaactaggagaatattacttacaaaatgcgtttctcgttgcttacacaaagaaagccccccagctgacctcgtcggagctgatggccatcaccagaaaaatggcagccacagcagccacttgttgccaactcagtgaggacaaactattggcctgtggcgagggagcggctgacattattatcggacacttatgtatcagacatgaaatgactccagtaaaccctggtgttggccagtgctgcacttcttcatatgccaacaggaggccatgcttcagcagcttggtggtggatgaaacatatgtccctcctgcattctctgatgacaagttcattttccataaggatctgtgccaagctcagggtgtagcgctgcaaacaatgaagcaagagtttctcattaaccttgtgaagcaaaagccacaaataacagaggaacaacttgaggctgtcattgcagatttctcaggcctgttggagaaatgctgccaaggccaggaacaggaagtctgctttgctgaagagggacaaaaactgatttcaaaaactcgtgctgctttgggagttggaagcggagctactaacttcagcctgctgaagcaggctggagacgtggaggagaaccctggacctatgagcaagggcgaggagctgttcaccggggtggtgcccatcctggtcgagctggacggcgacgtaaacggccacaagttcagcgtgtccggcgagggcgagggcgatgccacctacggcaagctgaccctgaagttcatctgcaccaccggcaagctgcccgtgccctggcccaccctcgtgaccaccctgacctacggcgtgcagtgcttcagccgctaccccgaccacatgaagcagcacgacttcttcaagtccgccatgcccgaaggctacgtccaggagcgcaccatcttcttcaaggacgacggcaactacaagacccgcgccgaggtgaagttcgagggcgacaccctggtgaaccgcatcgagctgaagggcatcgacttcaaggaggacggcaacatcctggggcacaagctggagtacaactacaacagccacaacgtctatatcatggccgacaagcagaagaacggcatcaaggtgaacttcaagatccgccacaacatcgaggacggcagcgtgcagctcgccgaccactaccagcagaacacccccatcggcgacggccccgtgctgctgcccgacaaccactacctgagcacccagtccgccctgagcaaagaccccaacgagaagcgcgatcacatggtcctgctggagttcgtgaccgccgccgggatcactcacggcatggacgagctgtacaagtaagtc